European Patent Application EP 4 279 594 A1, published November 22, 2023. Title: Multispecific antibody binding to ActRIIA,ActRIIB,and Fn14. Applicant: Astellas Pharma Inc. The sequence listing filed with the application follows.

SEQUENCE LISTING (18 sequences)

SEQ ID NO: 1 - DNA, 2160 bp, Artificial Sequence
  NMA_75E9S81.5_h1y_HC
  CDS (1)..(2160)
gaagtgcagctggttgaatctggcggcggattggttcagcctggcggatctctgagactgtcttgcgccgcctccagatccatctttgcctacggcaccatggcctggtacagacaggctcctggcaagggcagagaactggtggctacaatctctggcggaggcaccacctcctactccgactctgtgaagggcagattcaccatctccagagacaacggcaagtccaccgtgtacctgcagatgaactccctgagagccgaggacaccgccgtgtactactgcaacaagcggtctatcggcaccaacgatttctggggccagggcacactggtcacagtttctagcggaggcggaggatcaggtggcggtggaagtggtggtggcggaagtggcggcggtggatcaggcggtggcggatctgaagttcagctcgtggaaagtggcggaggactggtgcaaccaggtggaagtctgcggctgtcttgtgctgcctctggcttcaccctgaccaccaacgctctgatctggggcagacaagctccaggtgctgctcctggaaaaggccctgaatgggtggccggcatcagagctgatggcagaccttactacggcgactccatgaagggaagagtgaccatcagccgggatatcgccaagaacaccgcctatctccagatgaacagcctgcggcctgaggatacagctgtgtacttctgcgccaccagactggacgactctggcacctacgatagaggcagaggcacaaccgtgaccgtgtctagtggcggcggaggaagcggcggaggcggaagcgaagttcagttggttgagtcaggcggaggcctcgtgaaacctggcggtagcctcagactttcctgtgccgcttctggcatcaccttctccacctacggcatgaactgggtccgacaggcaccaggcaaaggactggaatgggtgtcctccatctcctctcggtccatccacatcagctacgccgacagcgtgaaaggccggttcaccatcagcagagataatgccaaaaactccctctacttgcagatgtcctctctgcgggccgacgatactgccgtgtattattgcgccagagacagaggcgccgctgccttcgattattggggcagaggaacactggtggccgtgtcctccgcttctaccaagggaccttctgtgttccctctggctccctccagcaagtctacttctggcggaacagctgccctgggctgcctggtcaaggattactttcctgagcctgtgacagtgtcctggaactctggcgctctgacatctggcgtgcacacctttccagctgtgctgcagtcctctggcctgtactctctgtcctccgtcgtgacagtgccttccagctctctgggcacccagacctacatctgtaatgtgaaccacaagccttccaacaccaaggtggacaagaaggtggaacccaagtcctgcgacaagacccacacctgtccaccatgtcctgctccagaagctgctggcggcccatccgtgtttctgttccctccaaagcctaaggacaccctgtacatcacccgcgagcctgaagtgacctgcgtggtggtcgatgtgtctcacgaggaccccgaagtgaagtttaattggtacgtggacggcgtcgaggtgcacaacgctaagaccaagcctagagaggaacagtacaacagcacctacagagtggtgtccgtgctgaccgtgctgcaccaggattggctgaacggcaaagagtacaagtgcaaggtgtccaacaaggccctgcctgctcctatcgaaaagaccatctctaaggccaagggccagcctcgggaaccccaggtttacacattgccaccttctcgggacgagctgaccaagaaccaggtgtccctgacctgtctcgtgaagggcttctacccctccgatatcgccgtggaatgggagtctaatggccagccagagaacaactacaagacaacccctcctgtgctggactccgacggctcattctttctgtactccaagctgacagtggacaagtccagatggcagcagggcaacgtgttctcctgcagcgtgatgcacgaggccctgcacaatcactacacccagaagtccctgtctctgtcccctggcaaa

SEQ ID NO: 2 - protein, 720 aa, Artificial Sequence
  Synthetic Construct
EVQLVESGGGLVQPGGSLRLSCAASRSIFAYGTMAWYRQAPGKGRELVATISGGGTTSYSDSVKGRFTISRDNGKSTVYLQMNSLRAEDTAVYYCNKRSIGTNDFWGQGTLVTVSSGGGGSGGGGSGGGGSGGGGSGGGGSEVQLVESGGGLVQPGGSLRLSCAASGFTLTTNALIWGRQAPGAAPGKGPEWVAGIRADGRPYYGDSMKGRVTISRDIAKNTAYLQMNSLRPEDTAVYFCATRLDDSGTYDRGRGTTVTVSSGGGGSGGGGSEVQLVESGGGLVKPGGSLRLSCAASGITFSTYGMNWVRQAPGKGLEWVSSISSRSIHISYADSVKGRFTISRDNAKNSLYLQMSSLRADDTAVYYCARDRGAAAFDYWGRGTLVAVSSASTKGPSVFPLAPSSKSTSGGTAALGCLVKDYFPEPVTVSWNSGALTSGVHTFPAVLQSSGLYSLSSVVTVPSSSLGTQTYICNVNHKPSNTKVDKKVEPKSCDKTHTCPPCPAPEAAGGPSVFLFPPKPKDTLYITREPEVTCVVVDVSHEDPEVKFNWYVDGVEVHNAKTKPREEQYNSTYRVVSVLTVLHQDWLNGKEYKCKVSNKALPAPIEKTISKAKGQPREPQVYTLPPSRDELTKNQVSLTCLVKGFYPSDIAVEWESNGQPENNYKTTPPVLDSDGSFFLYSKLTVDKSRWQQGNVFSCSVMHEALHNHYTQKSLSLSPGK

SEQ ID NO: 3 - DNA, 642 bp, Artificial Sequence
  STF_8-1_h1g_LC
  CDS (1)..(642)
gccatccagatgacccagtctccatcctctctgtccgcctctgtgggcgacagagtgaccatcacctgtagagcctctcaggccatctccaacgacctcggctggtatcagcagaagcctggcaaggctcccaagctgctgatctacgacgccatctctctgcagtctggcgtgccctctagattctccggctctggctctggcaccgactttaccctgacaatctccagcctgcagcctgaggacttcgccacctactactgcctgcaagacttcaactaccctcggacctttggccagggcaccaaggtggaaatcaagcggacagtggccgctccttccgtgttcatcttcccaccttccgacgagcagctgaagtccggcacagcttctgtcgtgtgcctgctgaacaacttctaccccagagaagccaaggtgcagtggaaggtggacaacgcactgcagtccggcaactcccaagagtctgtgaccgagcaggactccaaggacagcacctacagcctgtcctccacactgaccctgtccaaggccgactacgaaaagcacaaggtgtacgcctgcgaagtgacccatcagggcctgtctagccctgtgaccaagtctttcaaccggggcgagtgc

SEQ ID NO: 4 - protein, 214 aa, Artificial Sequence
  Synthetic Construct
AIQMTQSPSSLSASVGDRVTITCRASQAISNDLGWYQQKPGKAPKLLIYDAISLQSGVPSRFSGSGSGTDFTLTISSLQPEDFATYYCLQDFNYPRTFGQGTKVEIKRTVAAPSVFIFPPSDEQLKSGTASVVCLLNNFYPREAKVQWKVDNALQSGNSQESVTEQDSKDSTYSLSSTLTLSKADYEKHKVYACEVTHQGLSSPVTKSFNRGEC

SEQ ID NO: 5 - protein, 4 aa, Artificial Sequence
  Linker
GGGS

SEQ ID NO: 6 - protein, 4 aa, Artificial Sequence
  Linker
SGGG

SEQ ID NO: 7 - protein, 5 aa, Artificial Sequence
  Linker
GGGGS

SEQ ID NO: 8 - protein, 5 aa, Artificial Sequence
  Linker
SGGGG

SEQ ID NO: 9 - protein, 6 aa, Artificial Sequence
  Linker
GGGGGS

SEQ ID NO: 10 - protein, 6 aa, Artificial Sequence
  Linker
SGGGGG

SEQ ID NO: 11 - protein, 7 aa, Artificial Sequence
  Linker
GGGGGGS

SEQ ID NO: 12 - protein, 7 aa, Artificial Sequence
  Linker
SGGGGGG

SEQ ID NO: 13 - DNA, 1344 bp, Artificial Sequence
  STF_8-1_h1g_HC
  CDS (1)..(1344)
gaagtgcagctggttgaatctggcggcggactggttaagcctggcggatctctgagactgtcttgtgccgcttccggcatcaccttctccacctacggcatgaactgggtccgacaggctcctggcaaaggcctggaatgggtgtcctccatctccagccggtccatccacatctcttacgccgactccgtgaagggcagattcaccatcagccgggacaacgccaagaactccctgtacctgcagatgtccagcctgagagccgatgacaccgccgtgtactactgcgccagagatagaggcgccgctgccttcgattattggggcagaggaacactggtggccgtgtcctctgcttccaccaagggaccttccgtgtttcccctggctccttccagcaagtctacctctggtggcacagctgctctgggctgcctggtcaaggattacttccctgagcctgtgaccgtgtcctggaactctggcgctctgacatctggcgtgcacacctttccagctgtgctgcagtcctccggcctgtactctctgtcctctgtcgtgaccgtgccttccagctctctgggaacccagacctacatctgcaatgtgaaccacaagccttccaacaccaaggtggacaagaaggtggaacccaagtcctgcgacaagacccacacctgtccaccatgtcctgctccagaagctgctggcggcccttctgtgtttctgttccctccaaagcctaaggacaccctgatgatctctcggacccctgaagtgacctgcgtggtggtggatgtgtctcacgaggatcccgaagtgaagttcaattggtacgtggacggcgtggaagtgcacaatgccaagaccaagcctagagaggaacagtacaacagcacctacagagtggtgtccgtgctgaccgtgctgcaccaggattggctgaacggcaaagagtacaagtgcaaggtgtccaacaaggccctgcctgctcctatcgaaaagaccatctccaaggccaagggccagcctagggaaccccaggtttacaccttgccaccttctcgggacgagctgaccaagaaccaggtgtccctgacctgcctcgtgaagggattctacccctccgatatcgccgtggaatgggagtctaatggccagccagagaacaactacaagacaacccctcctgtgctggactccgacggctcattctttctgtactccaagctgacagtggacaagtccagatggcagcagggcaacgtgttctcctgcagcgtgatgcacgaggccctgcacaatcactacacccagaagtccctgtctctgtcccctggcaag

SEQ ID NO: 14 - protein, 448 aa, Artificial Sequence
  Synthetic Construct
EVQLVESGGGLVKPGGSLRLSCAASGITFSTYGMNWVRQAPGKGLEWVSSISSRSIHISYADSVKGRFTISRDNAKNSLYLQMSSLRADDTAVYYCARDRGAAAFDYWGRGTLVAVSSASTKGPSVFPLAPSSKSTSGGTAALGCLVKDYFPEPVTVSWNSGALTSGVHTFPAVLQSSGLYSLSSVVTVPSSSLGTQTYICNVNHKPSNTKVDKKVEPKSCDKTHTCPPCPAPEAAGGPSVFLFPPKPKDTLMISRTPEVTCVVVDVSHEDPEVKFNWYVDGVEVHNAKTKPREEQYNSTYRVVSVLTVLHQDWLNGKEYKCKVSNKALPAPIEKTISKAKGQPREPQVYTLPPSRDELTKNQVSLTCLVKGFYPSDIAVEWESNGQPENNYKTTPPVLDSDGSFFLYSKLTVDKSRWQQGNVFSCSVMHEALHNHYTQKSLSLSPGK

SEQ ID NO: 15 - protein, 489 aa, Artificial Sequence
  NMA_75E9.2_m10_HC
QVQLVESGGGLVQPGGSLRLSCAASRSIFAYGTMAWYRQAPGKQRELVATISGGGTTSYSDSVKGRFTISRDNGKSTVYLQMSSLKPEDTAVYYCNKRSIGTNDFWGQGTQVTVSSGGGGSGGGGSGGGGSGGGGSGGGGSQVQLVESGGGLVQTGGSLTLSCAASGFTLTTNALIWGRQAPGAAPGEGPEWVAGIRADGRPYYGDSMKGRVTVSRDIAKNTAYLQMTNLKPEDTAVYFCATRLDDSGTYDRGRGTQVTVSSVPRDSGCKPCICTVPEVSSVFIFPPKPKDVLTITLTPKVTCVVVDISKDDPEVQFSWFVDDVEVHTAQTKPREEQFNSTFRSVSELPIMHQDWLNGKEFKCRVNSAAFPAPIEKTISKTKGRPKAPQVYTIPPPKEQMAKDKVSLTCMITDFFPEDITVEWQWNGQPAENYKNTQPIMDTDGSYFVYSKLNVQKSNWEAGNTFTCSVLHEGLHNHHTEKSLSHSPGK

SEQ ID NO: 16 - protein, 442 aa, Artificial Sequence
  STF_8-1.2_m10_HC
EVQLVESGGGLVKPGGSLRLSCAASGITFSTYGMNWVRQAPGKGLEWVSSISSRSIHISYADSVKGRFTISRDNAKNSLYLQMSSLRADDTAVYYCARDRGAAAFDYWGRGTLVAVSSAKTTPPSVYPLAPGSAAQTNSMVTLGCLVKGYFPEPVTVTWNSGSLSSGVHTFPAVLQSDLYTLSSSVTVPSSTWPSQTVTCNVAHPASSTKVDKKIVPRDCGCKPCICTVPEVSSVFIFPPKPKDVLTITLTPKVTCVVVDISKDDPEVQFSWFVDDVEVHTAQTKPREEQFNSTFRSVSELPIMHQDWLNGKEFKCRVNSAAFPAPIEKTISKTKGRPKAPQVYTIPPPKEQMAKDKVSLTCMITDFFPEDITVEWQWNGQPAENYKNTQPIMDTDGSYFVYSKLNVQKSNWEAGNTFTCSVLHEGLHNHHTEKSLSHSPGK

SEQ ID NO: 17 - protein, 214 aa, Artificial Sequence
  STF_8-1.2_m10_LC
AIQMTQSPSSLSASVGDRVTITCRASQAISNDLGWYQQKPGKAPKLLIYDAISLQSGVPSRFSGSGSGTDFTLTISSLQPEDFATYYCLQDFNYPRTFGQGTKVEIKRADAAPTVSIFPPSSEQLTSGGASVVCFLNNFYPKDINVKWKIDGSERQNGVLNSWTDQDSKDSTYSMSSTLTLTKDEYERHNSYTCEATHKTSTSPIVKSFNRNEC

SEQ ID NO: 18 - protein, 714 aa, Artificial Sequence
  NMA_75E9STF8-1_m10_HC
QVQLVESGGGLVQPGGSLRLSCAASRSIFAYGTMAWYRQAPGKQRELVATISGGGTTSYSDSVKGRFTISRDNGKSTVYLQMSSLKPEDTAVYYCNKRSIGTNDFWGQGTQVTVSSGGGGSGGGGSGGGGSGGGGSGGGGSQVQLVESGGGLVQTGGSLTLSCAASGFTLTTNALIWGRQAPGAAPGEGPEWVAGIRADGRPYYGDSMKGRVTVSRDIAKNTAYLQMTNLKPEDTAVYFCATRLDDSGTYDRGRGTQVTVSSGGGGSGGGGSEVQLVESGGGLVKPGGSLRLSCAASGITFSTYGMNWVRQAPGKGLEWVSSISSRSIHISYADSVKGRFTISRDNAKNSLYLQMSSLRADDTAVYYCARDRGAAAFDYWGRGTLVAVSSAKTTPPSVYPLAPGSAAQTNSMVTLGCLVKGYFPEPVTVTWNSGSLSSGVHTFPAVLQSDLYTLSSSVTVPSSTWPSQTVTCNVAHPASSTKVDKKIVPRDCGCKPCICTVPEVSSVFIFPPKPKDVLTITLTPKVTCVVVDISKDDPEVQFSWFVDDVEVHTAQTKPREEQFNSTFRSVSELPIMHQDWLNGKEFKCRVNSAAFPAPIEKTISKTKGRPKAPQVYTIPPPKEQMAKDKVSLTCMITDFFPEDITVEWQWNGQPAENYKNTQPIMDTDGSYFVYSKLNVQKSNWEAGNTFTCSVLHEGLHNHHTEKSLSHSPGK